European Patent Specification EP 4 158 071 B1, published July 29, 2026. Title: PROBE FOR THE DETECTION OF BACTERIAL INFECTIONS. Applicant: Università degli studi di Udne. The sequence listing filed with the application follows.

SEQUENCE LISTING (5 sequences)

SEQ ID NO: 1 - DNA, 36 bp, Artificial sequence
  specific for Campylobacter species ieuni, upsaliensis, lari, coli
tagtggcgcacgggtgagtaaggtatagttaatctg

SEQ ID NO: 2 - DNA, 20 bp, Artificial Sequence
  universal forward primer P1V1
gcggcgtgcctaatacatgc

SEQ ID NO: 3 - DNA, 17 bp, Artificial Sequence
  universal reverse primer 518R
attaccgcggctgctgg

SEQ ID NO: 4 - DNA, 36 bp, Artificial Sequence
  negative control PR
cgtgcgccactacagattaccttaaactatctcacc

SEQ ID NO: 5 - DNA, 36 bp, Artificial Sequence
  negative control PE
aagacgcgcatctcttttttcaccagcgcgcttttc